European Patent Application EP 4 726 027 A1, published April 15, 2026. Title: A substance production of strains. Applicant: Synplogen Co., Ltd. Application JP. The sequence listing filed with the application follows.

SEQUENCE LISTING (14 sequences)

SEQ ID NO: 1 - DNA, 6092 bp, synthetic construct
  source 1..6092: mol_type = other DNA
aaaaggccttcttggccgcccttcccggtcgatatgaacagcttatttacataattcacgttattggtagttataaatgaaattcctaatatcggttatgaagtgaaattgaatttctacttgatctttctctctatttttgtaaaataaaattaagaatatttaaatattcaatgattcatttttgcagaaatcggaggaagaagaatatatgaaaacatttaacatttctcaacaagatccccccatattgttgtataagtgatgaaatactgaatttaaaacttagtttatatgtggtaaaatgttttaatcaagtttaggaggaattaattatgaagtgtaatgaataatgaatgtaacagggttcaattaaaagagggaagcgtatcattaaccctataaactacgtctgccctcattattggagggtgaaatgtgaatacatcctattcacaatcgaatttacgacacaaccaaattttaatttggctttgcattttatctttttttagcgtattaaatgaaatggttttgaacgtgtcattacctgatattgcaaatgattttaataaaccaccagcgagtacaaactgggtgaacacagcctttatgttaaccttttccattggaacagctgtatatggaaagctatctgatcaattaggcatcaaaaggttactcctatttggaattataataaattgtttcgggtcggtaattgggtttgttggccattctttcttttccttacttattatggctcgttttattcaaggggctggtgcagctgcatttccagcactcgtaatggttgtagttgcgcgctatattccaaaggaaaataggggtaaagcatttggtcttattggatcgatagtagccatgggagaaggagtcggtccagcgattggtggaatgatagcccattatattcattggtcctatcttctactcattcctatgataacaattatcactgttccgtttcttatgaaattattaaagaaagaagtaaggataaaaggtcattttgatatcaaaggaattatactaatgtctgtaggcattgtattttttatgttgtttacaacatcatatagcatttcttttcttatcgttagcgtgctgtcattcctgatatttgtaaaacatatcaggaaagtaacagatccttttgttgatcccggattagggaaaaatataccttttatgattggagttctttgtgggggaattatatttggaacagtagcagggtttgtctctatggttccttatatgatgaaagatgttcaccagctaagtactgccgaaatcggaagtgtaattattttccctggaacaatgagtgtcattattttcggctacattggtgggatacttgttgatagaagaggtcctttatacgtgttaaacatcggagttacatttctttctgttagctttttaactgcttcctttcttttagaaacaacatcatggttcatgacaattataatcgtatttgttttaggtgggctttcgttcaccaaaacagttatatcaacaattgtttcaagtagcttgaaacagcaggaagctggtgctggaatgagtttgcttaactttaccagctttttatcagagggaacaggtattgcaattgtaggtggtttattatccatacccttacttgatcaaaggttgttacctatggaagttgatcagtcaacttatctgtatagtaatttgttattacttttttcaggaatcattgtcattagttggctggttaccttgaatgtatataaacattctcaaagggatttctaaatcgttaagggatcaactttgggagagagttcaaaattgatcctttttttataacaggaattgggcatcaaataaaacgaaaggctcagtcgaaagactgggcctttcgttttatctgttgtttgtcggtgaacgctctcctgagtaggacaaatccgccgggagcggatttgaacgttgcgaagcaacggcccggagggtggcgggcaggacgcccgccataaactgccaggcatcaaattaagcagaaggccatcctgacggatggcctttttgcgtttctacaaactcttcctgtcgtcatatctacaattctacacagcccagtccagactattgaattgtatcacgtttttgatatcctaccaataacaaattgattggaggaatgcaaagtgaataatgaaccagtaaaacgtggtaagaagaacagatgggaattaaacctacctataatgacttatgtagtagctgatgattggattgataaactaggacacgaaacgtttactttatggttgaggttccatacttgggtagatagagaagatgaactccgagattatgatcgcatacctagaagttttgagaacatatataaaaagacactaggaatctcaaaaagtaagttttatagattgataaaacctttatgggaatatggattaatagacatcatagaatacgaagaatctaaccgtaattctactaaacctaaaaatataattgtttatgagtatcctttacacgaaatagaaagaaagtataaaccactagaaaaattaagagattgggataaagactataattccgtttctaaagaattaggtaaaacaggtggtagaccaaggaaaaaagatagtgaagaagaacccgaaaagaaacccgaagaagtaactaaaaagaaacgtaaatataagttaaaaagagttatccacaacggtttcaaaaatgaaacggtggagggtttcaaaaatgaaacggtggagggtttcaaaaatgaaacggtgaccgtttcaaaaataaaacccaataattattcaaatatctttaataacttatcaaatatttctactaatgtttcaaataatttattaattgatgatgatgaggaaatcgaaaatgaaccaactggtcgtacaataaataggtcattacttttttcacaagaagatattaaacaggcctatcaatttattaatagattttcagttatacagttacgtgaaaactttagctttgataaacactttgaagaacggttggtatgttatttatggaaagcagggatttctactttttacacgcacgaaatcagtaaaatgataaaaaaaatagcagactatgaaaaatctaaaaaaggtagattaaacccaatacgtgaccgagccttatatatggtaaatggtcttgtaatgaatagagcttcttcccaaagtgaacatgctacttataaactaaaccaatataaaaaacagaaggaacaggaaaaacaacaacaggagcaacaaagatcaagagtaccgttctataattggttggaggaaagagaagaacaaaccgaaggtcaactacccaccacttaagcggccgcaagcttgaagagctcttctttcagaacgctcggttgccgccgggcgttttttatgagatgtctcggcctgtttggccattaacgtgcaggtggatccagatctaagcttctatagaagcttggtaccgacgtctcggcctgtttggcccgccgcatccataccgccagttgtttaccctcacaacgttccagtaaccgggcatgttcatcatcagtaacccgtatcgtgagcatcctctctcgtttcatcggtatcattacccccatgaacagaaatcccccttacacggaggcatcagtgaccaaacaggaaaaaaccgcccttaacatggcccgctttatcagaagccagacattaacgcttctggagaaactcaacgagctggacgcggatgaacaggcagacatctgtgaatcgcttcacgaccacgctgatgagctttaccgcagctgcctcgcgcgtttcggtgatgacggtgaaaacctctgacacatgcagctcccgaagacggtcacagcttgtctgtaagcggatgccgggagcagacaagcccgtcagggcgcgtcagcgggtgttggcgggtgtcggggcgcagccatgacccagtcacgtagcgatagcggagtgtatactggcttaactatgcggcatcagagcagattgtactgagagtgcaccatatgcggtgtgaaataccgcacagatgcgtaaggagaaaataccgcatcaggcactcttccgcttcctcgctcactgactcgctgcgctcggtcgttcggctgcggcgagcggtatcagctcactcaaaggcggtaatacggttatccacagaatcaggggataacgcaggaaagaacatgtgagcaaaaggccagcaaaaggccaggaaccgtaaaaaggccgcgttgctggcgtttttccataggctccgcccccctgacgagcatcacaaaaatcgacgctcaagtcagaggtggcgaaacccgacaggactataaagataccaggcgtttccccctggaagctccctcgtgcgctctcctgttccgaccctgccgcttaccggatacctgtccgcctttctcccttcgggaagcgtggcgctttctcatagctcacgctgtaggtatctcagttcggtgtaggtcgttcgctccaagctgggctgtgtgcacgaaccccccgttcagcccgaccgctgcgccttatccggtaactatcgtcttgagtccaacccggtaagacacgacttatcgccactggcagcagccactggtaacaggattagcagagcgaggtatgtaggcggtgctacagagttcttgaagtggtggcctaactacggctacactagaaggacagtatttggtatctgcgctctgctgaagccagttaccttcggaaaaagagttggtagctcttgatccggcaaacaaaccaccgctggtagcggtggtttttttgtttgcaagcagcagattacgcgcagaaaaaaaggatctcaagaagatcctttgatcttttctacggggtctgacgctcagtggaacgaaaactcacgttaagggattttggtcatgagattatcaaaaaggatcttcacctagatccttttaaattaaaaatgaagttttaaatcaatctaaagtatatatgagtaaacttggtctgacagttaccaatgcttaatcagtgaggcacctatctcagcgatctgtctatttcgttcatccatagttgcctgactccccgtcgtgtagataactacgatacgggagggcttaccatctggccccagtgctgcaatgataccgcgagacccacgctcaccggctccagatttatcagcaataaaccagccagccggaagggccgagcgcagaagtggtcctgcaactttatccgcctccatccagtctattaattgttgccgggaagctagagtaagtagttcgccagttaatagtttgcgcaacgttgttgccattgctgcaggcatcgtggtgtcacgctcgtcgtttggtatggcttcattcagctccggttcccaacgatcaaggcgagttacatgatcccccatgttgtgcaaaaaagcggttagctccttcggtcctccgatcgttgtcagaagtaagttggccgcagtgttatcactcatggttatggcagcactgcataattctcttactgtcatgccatccgtaagatgcttttctgtgactggtgagtactcaaccaagtcattctgagaatagtgtatgcggcgaccgagttgctcttgcccggcgtcaacacgggataataccgcgccacatagcagaactttaaaagtgctcatcattggaaaacgttcttcggggcgaaaactctcaaggatcttaccgctgttgagatccagttcgatgtaacccactcgtgcacccaactgatcttcagcatcttttactttcaccagcgtttctgggtgagcaaaaacaggaaggcaaaatgccgcaaaaaagggaataagggcgacacggaaatgttgaatactcatactcttcctttttcaatattattgaagcatttatcagggttattgtctcatgagcggatacatatttgaatgtatttagaaaaataaacaaataggggttccgcgcacatttccccgaaaagtgccacctggatccacctgcacgt

SEQ ID NO: 2 - DNA, 1778 bp, synthetic construct
  source 1..1778: mol_type = other DNA
atcgatcggcaggtgatgtcaataacacctgcatcgggaatatgcaaagaggtgatcgcatggcgtttattttatccattggaacaagtctacctgcgtataatgtaaaccaagagaaagcggccgagttcgcccgctatatgtttcagcattcttttaaggatattgacaggctgttatcctcctttaaaaacgggcaaatccattcgagacagtttgttaagccgattgaatggtataaagaggggcacagctttgaagaaaaaaatcaaatatacatagaagaaacacttaaacacagcagagcggctgttcgtgagtgcctctctcatccggaattttttcaagaagccattccttatgagaaagtggaagctgtttttttcgtgtccagtacaggtctttccacaccgagtatcgaggcgcggcttatgaatgaacttccgttttctccatatacgaagcggattccgatttgggggcttggctgtgcaggaggagccagcggacttgcgcgtgcagccgaatactgcaaagcgtatcctgaggcttttgtgcttgtcatttctgccgagctgtgcagcctgacattccagccggaagataaaacaaaaagcaatctgatcggcacctcgctttttggtgacggcattgccgcagctttattatgcggagagaaggcggaccgcagggtgtcaaagctgaagcttgcgccgaagataatggacgcccaatctgttttgatgaaacaatcagaagatgtcatgggctgggactttaccgatcaaggattcaaagtcattttctcacgagacattccgaccttggtggaaaaatggctcaaaacaaatgtacagatttttttggacaaacataagctgtcattccatgatatcagtgtttttttggcgcatccaggcggaaaaaaagtgatcgatgcatacatcaaaagtctcgggctgtcgtcagaaaagctttcatctgcgcaaagcattttgcaaaagcacggaaatatgtcatcagccacaatcttgtatgtgatcaaagaccatctgcagaacggacataaaaaggaagctgaacgaggactgattggcgcattagggccgggtttctcatcagagttgctattattcagctgggaaaagggggcctgaggccttgatggccatcgagagaccaataataataggtctcaggaaaagggggcctgactcatgttttggttgttgatcgccattctcattgttcaaagagcagcagaaatggcagtggccaggcaaaacgaacaaaaggtaaagaagcaaggagcaattgaatttggcgagagccactatccgtatatcattacgatgcatatcctttttttcctgtccttaattgccgaggtgctgctgatgaataaacagccgtccagctggtggctcggtatcgctgcagtgattttaagcgtacagatcgtacggtattgggcgctttgttccttaggagcatattggaatacgaaaatccttgttgttccaggtgtagagcttgtaaaaaaaggtccatataaatggatgaaacatccaaactatgccgttgttatcctcgaaattttgctgattccgctgctttatcaagcatacgtcaccatgtgtctgttttccattttcaatgccgtgttgttaagcgtcagaattcgcgcagaggacaaagcattacaggaatacagcgtaaaatagaagaagaagtgtgaaaaagcgcagctgaaatagctgcgcttttttgtgtcataa

SEQ ID NO: 3 - DNA, 17669 bp, synthetic construct
  source 1..17669: mol_type = other DNA
atcgatcggcaggtgatgtcaataacacctgcatcgggaagaataaagggagaggtgaatgtgacttttatttcacaagtaaataaatggtttgttaatgctaatgttaactcagctgcaaagcttaggctattctgtattccatatgcaggcggtggtgcttccgccttttatgaatggagtcatttttttccaaaggaaattgaagtttgttcaattcaattacctggaagggaaaataggggggcggaagttccgctaacaaatttacaacagatagtagaaatagtagctgaggaaatacaaccattaataaatattccatttgcttttttggggcatagcatgggagcattaataagttttgaactggctcgcacaatacggcaaaagagtaatgttaatccggttcacttgtttgtttcagggcgacatgcacctcaaatcccatgtgcaaaacaagactatcatttacttcccgatgaacaatttatacaagaattgcgttcattgaatggaactccagagatagtattacaagacgcagagatgatgagtatattactcccaagacttcgggctgatttttctgtgtgtggctcctatcagtacaaaaacgacgagccttttgaatgcccaatcactgcttttggaggaaaaaatgataatggtgttacttatcaatcattagaagcctggagagagcaaaccaagagggaattttctgtgtgtatgtatccaggtgatcatttttttctttacgaaagcaaatatgaaatgattgagttcatgtgtaaacaattacgtttagtattagctcctaaaatataaggccttgatggccatcgagagaccaataataataggtctcaggaactattttttacagggggtatatatgttaaacagttctaaaagtatattgattcatgctcaaaataaaaatggaacgcatgaagaggagcagtatctctttgctgtgaacaacaccaaagcggagtatccacgtgataagacgatccatcagttatttgaggagcaggttagtaagaggccaaacaatgtagccattgtatgtgaaaatgagcaacttacctaccatgagcttaatgtgaaagccaatcaactagcacggatttttatagaaaaagggattggaaaagacactcttgttggaattatgatggagaaatctatcgatttatttataggcatattagccgttttaaaagctggtggagcatatgttccgattgatattgaatatcctaaggaaagaattcaatatattcttgatgatagtcaggcaagaatgctacttacccagaagcatttggttcatttaattcataatattcaatttaatgggcaagtggaaatttttgaagaagatactatcaaaattagagaaggaactaatctacatgtaccaagtaaatcaaccgatcttgcttatgttatttatacttctggtacaacaggcaatccaaaaggtacaatgctggagcataaaggaataagtaatctaaaggtatttttcgaaaatagtcttaacgtgactgaaaaggatagaattggtcaatttgccagcatctcttttgatgcatctgtatgggagatgtttatggctttgttaacgggggctagcctgtatattatcctgaaggatacaatcaatgattttgtgaagtttgaacaatacattaaccaaaaggaaatcactgttattacgttaccacctacctatgtagttcatcttgatccagaacgtattttatcgatacaaacgttaattacagcaggctcagctacctcgccttccttagtaaacaagtggaaggagaaagtaacttacataaatgcctatggccctacggaaacaactatttgtgcgactacatgggtagccaccaaagaaacaataggtcattcagttccaatcggagcaccaattcaaaatacacaaatttatattgtcgatgaaaatcttcaattaaaatcggttggtgaagctggtgaattgtgtattggtggagaagggttagcaaggggatattggaagcgaccggaattaacttcccagaagttcgttgataacccgtttgttccaggagagaagttgtataaaacaggagatcaggcaagatggctatctgatggaaatattgaatatctcggaagaatagataaccaggtaaagattagaggtcaccgagttgaactagaagaagttgagtctattcttctaaagcatatgtatattagcgaaactgcagtaagtgtgcataaagatcaccaagaacagccgtatttgtgcgcttattttgtatcggaaaagcatataccactagaacagttaagacaattctcatcagaagaactgccaacgtatatgatcccttcttattttatccagttagacaaaatgccgcttacatcaaatgggaagattgatcgaaagcagttgccggaacctgatttaactttcgggatgagggtagactatgaagcgccgcgaaatgaaatcgaggaaacgcttgttactatctggcaggatgtattaggtattgagaaaatcggtattaaagataatttctatgcattaggtggagattctattaaagcaatacaggttgctgctcgcctgcattcctaccaattaaagctagaaacaaaagatttattaaagtatccaacaatcgatcaactcgttcattatataaaagatagtaaaagaagaagtgagcaaggtattgtggaaggtgagattggacttacacctattcagcattggttctttgaacaacaatttacaaatatgcaccattggaaccaatcgtatatgttgtatagaccaaatgggtttgataaagagatcttgctaagggtatttaataaaattgttgagcatcatgatgcattacgtatgatatacaaacatcataacggaaagatcgtgcagataaatcgggggcttgaaggtacgttgtttgatttttatacctttgatttaactgcaaatgataatgagcaacaggtgatttgtgaagaatctgctcgattacaaaatagtataaacttggaagtaggccctctagtaaagatagcgctgtttcatactcagaatggagatcacctgtttatggctattcatcatttggttgtggatggtatttcttggaggattttgtttgaggatttggccacagcttatgaacaagcaatgcatcagcaaacgattgctttaccagagaaaacagattcatttaaggactggtctattgaattagaaaaatatgcgaacagcgaattattcctagaagaagctgaatattggcatcatttgaattattataccgagaacgttcaaattaagaaagattatgtcaccatgaacaataaacaaaagaatatacgttatgtaggaatggagttaacaatagaagagacagaaaaattattgaaaaatgtaaataaagcgtatcgaacagaaattaatgatattttattaacggcacttggctttgcactcaaagaatgggccgatattgataaaattgtaattaacttagagggacacggacgggaagaaatactggaacagatgaacattgcaaggacggtaggctggtttacttcccagtatcctgttgtacttgatatgcaaaaatcggatgatttgtcttatcaaatcaaattaatgaaagaaaatttacgcagaatacctaacaaaggaatcggatatgaaatttttaagtatttaacaactgaatatttacggcctgttttaccctttacattaaagccggaaattaactttaactacttaggacagttcgatacggacgtgaaaactgaattgtttactcgttctccttatagcatgggtaattcattaggaccagatggaaaaaataatttaagcccagaaggggaaagttattttgtactcaatattaatggttttattgaagaaggtaagcttcacatcaccttttcttataatgaacagcagtataaggaggataccattcagcaattgagccggagctataagcaacatcttttggccatcattgaacattgtgtacagaaggaagatactgagttaactccaagtgatttcagtttcaaggaacttgaattagaagagatggatgatattttcgatttgttggccgattcattaacgtaaggcctcgatggccatcgatgtcttcttattattatgaagacatggaacattattatgaggtgctagcatgagtacatttaaaaaagaacatgttcaggatatgtatcgtttatctcccatgcaggaaggcatgttgtttcacgcattacttgataaagataaaaatgctcacctggtacaaatgtctatcgcgatcgaaggtatcgtggatgtggagctgcttagtgaaagcttgaacatattgattgatagatacgatgtgtttagaacaacattcttacatgaaaaaattaaacaaccgcttcaggtagtgctaaaggaacggcctgttcagcttcaatttaaagacatatcatccttagatgaagaaaaaagagaacaggctattgagcagtataagtatcaagatggggaaacagtctttgatttaacaagagatcccttgatgagagtagctatttttcaaactggtaaggttaactaccaaatgatctggagcttccaccatattttaatggatggttggtgcttcaacattatatttaatgacttgttcaatatatatctgtcattaaaagagaagaaacctcttcagttagaggcggtgcaaccatataagcagtttattaagtggcttgaaaaacaagataaacaggaagcacttcgctactggaaagaacatttaatgaattatgatcaatcagtaacattacctaaaaagaaagcagctattaataatactacatatgaaccagcacagtttcgttttgcgtttgacaaagtgcttacccagcagctgcttcgtattgccaatcaaagccaagtaacactaaatattgtttttcaaacaatatgggggattgtacttcaaaaatacaattccactaatgatgttgtatatggctctgttgtatcaggccgtccttctgaaatatcgggaattgagaaaatggttggactatttattaatactcttccattacgtatccaaacgcaaaaagatcaatcatttattgaattagtaaagactgttcatcaaaacgtccttttctcgcaacagcatgagtattttccattgtatgaaatacaaaatcatacagaattaaaacagaatctgattgatcatattatggtaattgaaaattatcctttagtagaagaattgcaaaagaatagtatcatgcaaaaagtagggtttacagttcgtgatgtcaaaatgtttgaaccaactaattatgatatgacagttatggttttacctcgtgatgaaattagtgtccgactcgattataacgcagccgtttatgatatagatttcataaaaaaaattgaaggtcacatgaaagaagtggctttatgcgtggcaaataatccacatgtgttagtacaggacgttcctctgcttacaaagcaagaaaaacaacatttattggtagagctgcatgattcgataacagagtatcctgataagacgattcatcagttatttacagaacaggtagaaaaaacaccagagcatgtggcagttgtattcgaagatgagaaagtgacctatagagagctgcatgagagatctaatcaattagccagattcttaagagaaaaaggcgtaaaaaaagaaagcatcataggcattatgatggagcgttcagttgaaatgattgttgggatcttagggattttaaaagctggtggagcttttgtgcctattgatcctgaatatccaaaagaaagaatcggctatatgttagattctgtacggctagtacttacacaacgccatttaaaggataaatttgcttttacgaaagaaacgatagtaattgaagatccaagtatttcacacgagttaactgaagaaatagattatattaatgaatcagaggacttgttttatattatttatacatcaggaacaacaggtaaaccaaaaggggttatgctagagcacaaaaacatcgttaatctgcttcattttactttcgagaaaacaaatatcaactttagtgacaaagtattacagtatacaacatgcagttttgacgtgtgttaccaagaaattttttcgacgctcttgtctggagggcaattatatcttattaggaaagaaactcaacgcgatgtagagcaattatttgatttagtaaaacgtgaaaatattgaagtattatcctttcctgtggcttttctaaaatttattttcaatgaaagagaatttatcaatcgttttccaacttgcgtgaaacatattatcacagcaggagaacaattagtagttaacaatgagtttaaacgttatttgcatgaacataacgtacatttacacaatcattatggtccatcagaaacgcatgttgttaccacctatactattaatcctgaagctgaaattcctgaattaccaccgataggaaaacctatctccaatacatggatttatattttggatcaagaacaacaactacaaccacaaggaattgtaggagagttatatatttcgggcgcaaatgttggaagaggatatttgaataatcaagaattaacggcagaaaaattctttgcagatccctttaggccaaacgaacggatgtaccgaacaggggatttagcaaggtggttgccagacggaaatatcgaatttttaggaagggccgatcatcaggtgaaaattagggggcatcgaatagagcttggtgagatcgaggcacaattattaaattgtaagggtgtaaaagaagctgttgttatcgataaagcggatgataaaggcggaaaatatttatgtgcctatgttgttatggaagtagaagtaaatgactctgagcttcgagaatatttggggaaagctttgcctgattatatgatcccgtcgttctttgttccgttggatcagctgccgcttacaccaaacggaaaaatagacagaaaatctcttccgaatctagaggggattgtgaatacaaacgcaaaatatgtagtacctacaaatgagctggaagaaaaattggctaaaatctgggaagaagtacttgggatttctcagatcggtatacaagacaatttcttttcgttaggcgggcattctcttaaagccattacgcttatttcccgtatgaacaaagagtgtaatgtagacattcctctacgtttgttatttgaagcaccaaccattcaggaaatctctaattatataaacggggcaaagaaagaaagctatgttgccattcagcctgtaccagaacaagagtactatcctgtatcatcagttcaaaaaagaatgtttattcttaatgaatttgatcgttcaggtacggcctataatttacctggtgttatgtttctagatggaaaattgaactaccgacaattggaagcagcggtaaaaaaattagttgagcgacatgaagcgctgcgtacttcctttcattcaattaatggggaaccagttcagcgggtgcatcaaaatgtagaactgcagattgcttattcagagtcaacggaagatcaggtggagcgaattattgcggaatttatgcaaccatttgctcttgaagttgctccgttacttcgtgtaggtcttgttaaattggaggcagaacgtcatctatttataatggatatgcatcatatcatctcggatggggtatccatgcagatcatgattcaagaaattgctgatttgtataaagaaaaggaacttcctacgttaggcattcaatataaagactttactgtttggcataatcgcttgcttcaatcggatgttattgaaaaacaagaagcttactggctgaacgtatttgcagaagagattccagtattgaatctaccgaccgattacccaagaccaaccattcaaagctttgatggtaaaagatttacattcagtacaggaaagcagcttatggatgatttatacaaggtggcaacagaaacaggaacaacactatatatggttttacttgctgcgtataatgttttcttatcgaagtattccgggcaagatgacatcgttgtaggaacaccgattgctggtaggtcccatgctgatgtggaaaatatgctggggatgtttgtaaatacattagcaataagaagtcgtttaaataatgaggatacttttaaagattttttagcaaatgtaaaacaaacggctttgcatgcctatgaaaatccagattacccatttgatacgcttgtcgaaaagttgggtatacagagagatttaagtagaaatccattatttgatacgatgtttgttttgcaaaatacggatagaaagtcttttgaggttgaacagataacgattacaccatatgttccaaatagcagacattctaaatttgatcttacattagaggttagcgaagaacaaaatgagattttattatgcctagaatattgcactaaattatttacggataaaacagttgaaagaatggctggtcattttttacagatcttgcatgcaattgttgggaacccaacgattataatatcagaaatcgagatattgtctgaagaagaaaaacaacatattttattcgagttcaacgatacgaaaaccacatatccacatatgcaaacaattcaaggattatttgaggaacaggtggagaaaacgcccgaccatgttgcagttggatggaaagaccaaacattaacgtatcgggaacttaacgaaagagcgaatcaggtcgcaagagtcttacggcaaaaaggagtccaacccgataatatcgtgggattgctggttgagcgttcacctgaaatgctcgtgggtatcatgggaattcttaaagcagggggagcttatttacctcttgatccggagtacccagcggatagaatttcgtacatgatacaagattgtggtgtacgcattatgcttacccaacagcatcttttatctttagtacatgatgaatttgattgtgttattttggatgaggacagtttgtacaagggggattcttccaatttggctccggttaaccaggccggggatttagcctacatcatgtacacttctggttctacaggaaagcctaaaggtgttatggtagaacatcgaaatgtgattcgccttgtgaaaaatacaaattatgttcaggtccgcgaggacgatcgtataatacagaccggagcaattggattcgatgcactgacatttgaagtttttggctcattgctgcatggagctgaattgtatcctgttactaaagacgtgctattagatgcagagaaactacacaaatttttacaagcgaatcaaattacgattatgtggttaacttctccgttatttaaccaattgtcacaaggaaccgaagagatgtttgctggccttcgctccctaattgtaggtggagatgccttgtctccgaaacacatcaataatgtaaagcgaaaatgccctaatctgactatgtggaacggttacggcccaacagaaaacaccactttttctacatgctttcttattgataaagaatatgatgacaatattccgatagggaaggccattagtaattcaacagtgtatatcatggaccggtatggccagcttcagccggtgggtgtaccaggagaattatgtgtaggaggggatggggttgccaggggatatatgaatcagcctgcattaacagaagagaagtttgtcccaaatccattcgctcctggtgagagaatgtatcgcacgggggatttggcaagatggttgcctgatggaacaattgagtatttaggtcgtattgatcagcaagtgaaaatcaggggctaccgtattgaaccgggagagattgaaacgcttcttgtgaagcacaaaaaagtcaaagaatcggtaatcatggtagtagaggataataatggacaaaaggctctatgcgcttattacgttccggaagaagaagtaacggtatctgaactgagggaatatatagctaaagagttgcctgtttacatggttccagcctattttgtacagattgaacaaatgcctcttacacagaacggtaaagtaaatcgaagcgcgttaccaaaaccagatggtgaatttggtacagcaaccgaatatgtagcgcctagcagcgacattgaaatgaagctggcagagatttggcataatgtgttaggggtaaacaaaatcggggtactggataacttctttgaattaggtggtcattcattaagagctatgacaatgatttcccaggtacataaagagttcgacgttgaattgccattaaaagtgttatttgaaacaccaacgatctctgcattagctcaatacattgctgatggagaaaaaggaatgtacctggccattcaacctgttaccccgcaggattactatccagtatcatctgcgcaaaagaggatgtacatcctttatgaatttgaaggggctggcattacctataatgtacctaatgtaatgtttatagaaggaaagctggattatcagcgctttgaatacgctataaaaagtttggtaaatcgacatgaggcgcttcgaacgtctttctattcgcttaatggagaaccagttcagcgtgtacatcaaaatgtagagctacagattgcttattcggaggcgaaagaagatgagatagagcaaattgtagaaagctttgttcaaccatttgaccttgaaatagctccgctgcttcgcgtagggcttgttaaattggcatcggatcgctatttattcctaatggatatgcatcatattatctcagatggtgtatcaatgcaaattataacaaaagaaattgccgacttatataaaggaaaagagcttgctgaactgcatattcagtataaagattttgctgtatggcaaaacgaatggtttcaatctgacgctcttgaaaaacagaaaacgtattggttgaacacctttgcagaggatattccggttttaaatttgtcaactgattatccaagaccgacaattcaaagttttgaaggagatattgtcacgtttagtgcagggaagcaacttgcggaagaattgaaacgcctggctgcagaaacagggacgactttgtatatgcttctgttagcggcgtacaatgtacttttacacaaatactcgggacaggaagaaattgtagtaggaacgcctattgccgggcgatctcacgcagatgtggaaaatattgttgggatgtttgtcaatacgcttgcattgaaaaatacccctatagccgtacgcaccttccacgaattcctgttggaagtaaaacaaaatgctttagaagcttttgaaaatcaagactatccatttgaaaatttgatagagaagctgcaagtgcgtcgcgacttaagtcgcaatccattatttgatacaatgtttagcctaagcaatattgacgaacaagtagagatagggattgagggattgaacttcagcccatatgaaatgcagtattggattgcaaaatttgatatttcattcgatattttagaaaagcaagatgacattcaattttattttaactattgcacgaatctgtttaaaaaagaaacgatagaacgattagcgacacactttatgcatattttacaggagattgttattaatcctgagattaagttatgtgaaattaatatgctgtccgaagaagaacagcagcgtgtcctgtatgactttaatggcacagatgcaacctacgctacgaataaaatattccatgagttatttgaagaacaggttgaaaaaacaccagatcatatagcggtgatagatgaaagagaaaagctttcctatcaggagcttaatgcgaaagcgaatcagctggcacgagtgctgcgccaaaaaggagtacagcctaatagcatggtaggtattatggtagatcgctcactcgacatgattgtaggaatgcttggggttttaaaagcaggaggagcatatgtgcctatcgatatagactatcctcaggaacggattagctacatgatggaagatagtggtgcagcgctcttgttaacacaacaaaagttgacacagcaaattgcgttttctggtgacattttgtatcttgaccaagaagaatggcttcatgaggaagcttcaaatttagaacccatcgctcgtccgcaggatatagcctatatcatttacacttctggtacaaccggaaagccaaaaggtgtgatgattgagcatcaaagctatgtgaatgtagcaatggcatggaaagatgcctatcggttagatacattcccggtccgtttgcttcagatggctagctttgcctttgacgtatctgcgggtgattttgccagagcactacttacaggtgggcaattaattgtatgtccaaatgaagtaaagatggacccagcttctttatatgccattattaagaaatatgacattactatttttgaagcaacgcctgctctagtgattccattgatggagtatatttatgaacagaagctggatattagccagttacagattctgattgtcggatcggacagttgttcgatggaggactttaaaaccttggtttcccgttttggttcaactatacgtattgtgaatagctatggagtaaccgaagcgtgcattgattctagctattatgaacaaccgctttcttcgttacatgtaacaggaactgtaccgattggaaaaccgtacgctaacatgaaaatgtatattatgaatcaatatttgcagattcagcctgtaggtgtaattggagaattatgtattggaggagccggggttgcccgtggatatttaaatagaccggacttaacagcagaaaagtttgtccctaatccttttgttccaggtgaaaagctgtatcgaacaggcgacttggcaagatggatgccggatgggaatgttgagtttcttggtcgaaatgaccatcaggtgaaaatcagagggattcgaatcgagcttggagaaatcgaagcacaactgcgtaaacatgatagcataaaagaagcaactgtgatcgcaagagaagatcacatgaaagagaaatatttatgtgcgtatatggtgaccgaaggagaagtaaatgtagctgaactgcgtgcgtatctagcaaatgatctgcctgcggcaatgattccgtcatattttgtatcgctcgaagcaatgccacttactgctaatggaaaaattgataagcgatctttaccagagcccgatggttccatatcgataggaacagaatatgtagctccgcgtaccatgcttgagggaaaactagaagagatatggaaagatgtattgggtttacagcgtgttggcattcacgatgacttctttacaataggtggccattcattgaaggctatggctgttatttcgcaagttcataaagaatgccagactgaagttcctctgcgtgtcttatttgaaacacctaccattcaaggactggctaaatatatagaggaaacggacacagagcaatatatggctattcagccggttagcggacaggactattatccagtatcatcagcacaaaagagaatgtttattgttaatcaatttgatggagtaggaattagctacaatatgccttccatcatgctgattgaaggaaaacttgagcgaacacgcttggaatcagcatttaaaagattgatagaacgacatgagagccttcgaacatcttttgaaataataaatggtaagcctgtacagaagattcatgaggaagttgatttcaatatgtcctatcaggtggcttctaatgaacaagtagagaagatgatcgatgagttcattcagcctttcgatttaagtgttgcaccgctgcttcgtgtggaacttttaaaattggaagaggaccgtcatgtgcttatatttgatatgcatcatattatctcagatggtatatcttccaatattttgatgaaagaattaggagaactatatcaaggtaatgctttaccagaacttcgtattcaatacaaggatttcgctgtatggcaaaatgagtggttccagtcagaagcctttaaaaagcaagaagaatactgggtaaatgttttcgcagatgaacgcccgattctggatataccgacggattatccaaggccgatgcaacaaagctttgatggtgctcaacttacatttggaaccggaaagcagcttatggatgggttatacagggtagcaacggaaacgggaacaacgctttatatggttttgcttgcggcatataatgttcttctttccaaatattctggtcaagaagatattattgtagggacaccgattgtgggtagatcccatactgaccttgagaatattgtcgggatgtttgtcaacacgttagcaatgagaaataaaccggaaggagaaaagacgttcaaagcatttgtatcagaaataaagcagaatgcactagcggcttttgagaatcaggattatccatttgaggagcttatcgaaaaactagagatacaaagggacttaagcagaaatccattatttgatacgctctttagccttcaaaacataggtgaagaatcatttgaactagccgaattaacatgcaaacctttcgatttggtaagcaaattagagcatgccaagtttgatctgagtcttgtggcagtagaaaaagaggaagaaattgcatttgggcttcaatactgcacaaaactgtataaggaaaaaacagttgaacaactggctcaacattttattcaaatagtaaaagcaattgtagaaaatccagatgtcaaattatctgatattgatatgttatctgaagaagagaagaaacaaatcatgcttgagttcaatgatacgaaaatacaatatccgcagaatcaaacaatacaggaattgtttgaggagcaagtgaagaaaacacctgaacatatagcaatcgtatgggaagggcaagcattaacctatcatgagctaaatataaaagctaatcagttagctcgtgtattacgagaaaaaggggtaacccctaatcatcctgtagcgattatgacggaacgctcattagagatgatcgtaggtatctttagtattttgaaagcaggaggagcatatgttccaattgatccagcctatccacaagaacgtattcaatacttgcttgaagatagcggagcgacgctactgcttactcagtcacatgtattaaataaattaccggtcgatatcgaatggttggatcttacagatgaacaaaactatgtagaagatggtaccaatcttccatttatgaatcagtcaacagatcttgcctatattatttatacatccggtacaacaggcaagcctaaaggggttatgattgaacatcaaagcatcatcaactgcctgcaatggcggaaggaagaatacgaatttggaccaggggatacggctctacaagtgttttcctttgcttttgatggatttgtagcaagtttgtttgctccgattcttgctggtgcaacgtctgttctccctaaggaggaagaagcaaaagatccagttgcattgaaaaaactgatcgcatcagaagagattacacattactacggtgtgcctagtttgtttagtgccattcttgatgtttcttctagtaaggatttgcaaaatttacgctgcgtcactttgggaggagagaaattaccggctcaaattgttaaaaaaatcaaagaaaaaaataaagaaattgaagtcaacaacgaatatgggcctactgaaaatagtgtagtaactactattatgcgcgatatacaggtagaacaagagattactattggtcgcccattatctaacgtagatgtatatattgtcaattgtaatcatcaattacaaccagtaggtgtagtaggggaattatgtattggtggacagggacttgcaagaggatatttgaataaaccagagcttacagcagataaatttgttgtaaatccattcgtacctggtgaacgtatgtacaaaaccggtgaccttgcaaaatggcgctcagatggaatgattgaatatgtggggcgtgttgatgaacaagtaaaagtaagaggatatcggattgagcttggtgaaattgaatcagctatcctagaatacgaaaaaattaaggaagcggtagttatggtttcggagcatactgcatctgaacagatgttatgtgcttatattgtaggggaagaagatgtactgactctggacttaagaagctatctagcaaaattactaccaagttatatgattccaaactattttatccaattggatagtattccgcttacaccaaacggtaaagtggatcgtaaagcattgcctgaacctcaaaccattggcttaatggcaagggagtatgttgcaccaaggaatgaaatcgaagcacagctagtactcatttggcaagaggtattaggaatagaactgatcggtattaccgataatttctttgaattaggagggcattctttaaaggcaacgcttttagttgcaaaaatttacgagtacatgcaaatagagatgccattaaatgttgtgtttaaacattcaactattatgaaaatagcggaatatattacacatcaagaatcagaaaataatgtacatcagcctattttggtaaatgtagaagcagatagagaggcgctatctcttaacggcgagaagcaaagaaaaaatatagagctacctattctgctaaacgaagaaacagatcgaaacgtattctgcttcgcgcccattggtgcacaaggtgttttttataaaaagcttgctgaacaaatccctactgcatccttgtatggctttgacttcattgaagatgatgatcgaattcagcaatatattgaatcgatgattcaaactcagtcagacggacaatatgtgctaattggttattcttcaggagggaacctggcttttgaagtagcaaaagaaatggaaaggcaaggatatagtgtatctgatttggtcttgttcgatgtttactggaagggaaaagtattcgagcaaacaaaagaagaagaagaagaaaacataaaaataataatggaagaattaagggaaaatccaggaatgttcaatatgacacgagaggattttgaactgtattttgcgaatgaatttgtgaaacaaagtttcacacggaaaatgcgcaaatacatgagtttttatacgcagttagttaattatggggaagtagaagctacaattcaccttatacaagcagaatttgaggaagaaaaaattgacgaaaacgaaaaagccgacgaagaagaaaaaacatatctagaggaaaaatggaatgaaaaagcatggaacaaagcagcaaaaagatttgtaaaatataacggatatggcgctcattctaacatgctaggaggtgatggtttagagagaaattcctctatccttaaacagatactacaagggacatttgtagtaaaataaaagaagaagtgtgaaaaagcgcagctgaaatagctgcgcttttttgtgtcataa

SEQ ID NO: 4 - DNA, 358 bp, synthetic construct
  source 1..358: mol_type = other DNA
aagaagaagtgtgaaaaagcgcagctgaaatagctgcgcttttttgtgtcataatcctaatatatacatacgccctgaaaaagaataattaaaattaaaaatctttaatgaaaataaaaaaagtctgttcgtgtcgaattttgtcgtatataatcaaatgaaataaaaaactttggttcgaaagtcttgatttaaaaggatttttagtaggataatagctttattaaatatttataaaatgctgttatttcggtagtttccaagacattactgactataagaactaattcttacaatcaatagtaaacaaaatgattgacgattattggaaaccttgttatgctatgaaggtaaggat

SEQ ID NO: 5 - DNA, 358 bp, synthetic construct
  source 1..358: mol_type = other DNA
aagaagaagtgtgaaaaagcgcagctgaaatagctgcgcttttttgtgtcataatcctagattaggattgcgagcagcaaaacatcaaaggttgtcggaaagaaaatggttctgattccttgaaaaatcgtaatgggaataatcacttgtgcggatacaagccgaatttgccttacccatggcggcagcgaataagagctgaaacgtttcttcacggtgcatcctcctctacgcatttacaagcatcatatgtaaacttgggcaataggtgcctgcccatctgtatagaaagcggtgtttttggaaaagatgattgacgaatcaaaaacacttttactataataaagaacataaataa

SEQ ID NO: 6 - DNA, 358 bp, synthetic construct
  source 1..358: mol_type = other DNA
aagaagaagtgtgaaaaagcgcagctgaaatagctgcgcttttttgtgtcataatccttgaagtaaaagtgattgcggttgaaggggatcaagtgaagcttggaattgacgccccaaagcatattgatattcacaggaaagaaatttacttgaccattcaggaagaaaataaccgtgcagcagcgttatccagcgatgtgatctccgcattatcctcacaaaaaaagtgaggatttttttatttttgtattaacaaaatcagagacaatccgatattaatgatgtagccgggaggaggcgcaaaagactcagccagttacaaaataagggcacaaggacgtgccttaacaacatattc

SEQ ID NO: 7 - DNA, 358 bp, synthetic construct
  source 1..358: mol_type = other DNA
aagaagaagtgtgaaaaagcgcagctgaaatagctgcgcttttttgtgtcataatccttgcggaagtaaacgaagtgtacggacaatattttgacactcacaaaccggcgagatcttgtgttgaagtcgcgagactcccgaaggatgcgttagtcgagatcgaagttattgcactggtgaaataataagaaaagtgattctgggagagccgggatcacttttttatttaccttatgcccgaaatgaaagctttatgacctaattgtgtaactatatcctattttttcaaaaaatattttaaaaacgagcaggatttcagaaaaaatcgtggaattgatacactaatgcttttatatag

SEQ ID NO: 8 - DNA, 358 bp, synthetic construct
  source 1..358: mol_type = other DNA
aagaagaagtgtgaaaaagcgcagctgaaatagctgcgcttttttgtgtcataatcctgacgctcttcgcaagggtgtctttttttgcctttttttcggtttttgcgcggtacacatagtcatgtaaagattgtaaattgcattcagcaataaaaaaagattgaacgcagcagtttggtttaaaaatttttatttttctgtaaataatgtttagtggaaatgattgcggcatcccgcaaaaaatattgctgtaaataaactggaatctttcggcatcccgcatgaaacttttcacccatttttcggtgataaaaacatttttttcatttaaactgaacggtagaaagataaaaaatat

SEQ ID NO: 9 - DNA, 358 bp, synthetic construct
  source 1..358: mol_type = other DNA
aagaagaagtgtgaaaaagcgcagctgaaatagctgcgcttttttgtgtcataatccttattgagtggatgattatattccttttgataggtggtatgttttcgcttgaacttttaaatacagccattgaacatacggttgatttaataactgacaaacatcaccctcttgctaaagcggccaaggacgctgccgccggggctgtttgcgtttttgccgtgatttcgtgtatcattggtttacttatttttttgccaaagctgtaatggctgaaaattcttacatttattttacatttttagaaatgggcgtgaaaaaaagcgcgcgattatgtaaaatataaagtgatagcggtacc

SEQ ID NO: 10 - DNA, 358 bp, synthetic construct
  source 1..358: mol_type = other DNA
aagaagaagtgtgaaaaagcgcagctgaaatagctgcgcttttttgtgtcataatcctctaaccctacataagtaccttcttttgtttcaatgttactgtctggcgatacatcttcaccttgactcttttgactattaaccccgcaacccgaaagaagcaatataaagaacagtaaagcaataaattttttcatttttttcacctcattatattttatcgtcaacctattttatattttaaagaaaaattaagaaacaatgaaacttttttttataaaaaacgactattttaggatttcattcttgtattaaatagagttgtatttattggaaatttaactcataatgaaagtaattt

SEQ ID NO: 11 - DNA, 358 bp, synthetic construct
  source 1..358: mol_type = other DNA
aagaagaagtgtgaaaaagcgcagctgaaatagctgcgcttttttgtgtcataatccttatgggaagtgctccgtaatacgctgacaagagagaaagggcttggaggtattgaaacaagaggagttctgagaattggtatgccttataagtccaattaacagttgaaaacctgcataggagagctatgcgggttttttattttacataatgatacataatttaccgaaacttgcggaacataattgaggaatcatagaattttgtcaaaataattttattgacaacgtcttattaacgttgatataatttaaattttatttgacaaaaatgggctcgtgttgtacaataaatgtagtg

SEQ ID NO: 12 - DNA, 358 bp, synthetic construct
  source 1..358: mol_type = other DNA
aagaagaagtgtgaaaaagcgcagctgaaatagctgcgcttttttgtgtcataatccttcgatatatcgcgtctattccggcttccggctatcacccgaagataaacagcccaggggtcacagatgaagtactgaagaaaatgaggaacggtttgattaaggtaaggccgtatacagtcaatcgtccggaagatatgaagcgtctcattgaagcgggagcagacggcatgtttaccgactttccagaaaaggcttcggcattgctgaaaaatgaatagttgttagaaggaggctgtttgacgcagccttcttttttcattcattcatgcccgtttcaaagcatacattcatagaagac

SEQ ID NO: 13 - DNA, 358 bp, synthetic construct
  source 1..358: mol_type = other DNA
aagaagaagtgtgaaaaagcgcagctgaaatagctgcgcttttttgtgtcataatcctagatgcccctgcacctatccctaaccgtatggaacaggcaagacgggaagcggaagaaagacgcagggaaacagcaagaaacctgaaagggctggaacgagatcttgctgctgccaaacaaaaaacagtatacacaaaacaaaaaatgcttcaggtgaataaagacaccgtcgtacaggggatcgttctaggagaggtgttcggacctccacgggcgaaaaaacctcaccgtacgatgcgcccggcccgtaaaaattaaagtgttagaacctcctttcaaatcatacatatgagatgaaa

SEQ ID NO: 14 - DNA, 358 bp, synthetic construct
  source 1..358: mol_type = other DNA
aagaagaagtgtgaaaaagcgcagctgaaatagctgcgcttttttgtgtcataatccttgcccccctccaccattattgggctatagccaagcggtaaggcaacggactttgactccgtcatgcgttggttcgaatccagctagcccagtcacagacacctttgatcaaaaggtgtcttttttcttttcggaaaaatcattccaacttctaactgttcagtctgtataataattttaaaaatatgttaaggtagtttattcacgaattaccatctacaccctgccaaaaatttgataaacttattttataaaaaaattgaaaccttttgaaacgaagctcgtatacatacagaccggt